European Patent Application EP 4 169 952 A1, published April 26, 2023. Title: ANTI-TROP2 ANTIBODY. Applicant: BAILI-BIO (CHENGDU) PHARMACEUTICAL CO., LTD. Application EP21828738.1. The sequence listing filed with the application follows.

SEQUENCE LISTING (40 sequences)

SEQ ID NO: 1 - protein, 8 aa, 2 Ambystoma laterale x Ambystoma jeffersonianum
GYTFTSFD

SEQ ID NO: 2 - protein, 7 aa, 2 Ambystoma laterale x Ambystoma jeffersonianum
IFPGDGN

SEQ ID NO: 3 - protein, 11 aa, 2 Ambystoma laterale x Ambystoma jeffersonianum
VRGEALYYFDY

SEQ ID NO: 4 - protein, 8 aa, 2 Ambystoma laterale x Ambystoma jeffersonianum
GYTFTDHV

SEQ ID NO: 5 - protein, 8 aa, 2 Ambystoma laterale x Ambystoma jeffersonianum
IYPGSDNS

SEQ ID NO: 6 - protein, 18 aa, 2 Ambystoma laterale x Ambystoma jeffersonianum
AREGYGYGKNGVGYAMDY

SEQ ID NO: 7 - protein, 6 aa, 2 Ambystoma laterale x Ambystoma jeffersonianum
QDINKY

SEQ ID NO: 8 - protein, 3 aa, 2 Ambystoma laterale x Ambystoma jeffersonianum
STS

SEQ ID NO: 9 - protein, 8 aa, 2 Ambystoma laterale x Ambystoma jeffersonianum
LQYDDLFT

SEQ ID NO: 10 - protein, 6 aa, 2 Ambystoma laterale x Ambystoma jeffersonianum
QSVSND

SEQ ID NO: 11 - protein, 3 aa, 2 Ambystoma laterale x Ambystoma jeffersonianum
YAS

SEQ ID NO: 12 - protein, 9 aa, 2 Ambystoma laterale x Ambystoma jeffersonianum
QQDYSSPWT

SEQ ID NO: 13 - protein, 137 aa, 2 Ambystoma laterale x Ambystoma jeffersonianum
MGWSWVFLFLLSVTAGVHSQVQLQQSGAELVKPGASVKLSCKASGYTFTSFDINWVRQRPEQGLEWIGWIFPGDGNTKSNEKFKGKATLTTDKSSSTAYMQLSRLTSEDSAVYFCVRGEALYYFDYWGPGTTLTVSS

SEQ ID NO: 14 - protein, 126 aa, 2 Ambystoma laterale x Ambystoma jeffersonianum
MRPSIQFLGLLLFWLHGAQCDIQMTQSPSSLSASLGGKVTITCKPSQDINKYIAWYQHKPGKGPRLLIHSTSTLQPGIPSRFSGSGSGRDYSFTISNLEPEDIATYYCLQYDDLFTFGSGTKLEIK

SEQ ID NO: 15 - protein, 143 aa, 2 Ambystoma laterale x Ambystoma jeffersonianum
MEWRIFLFILSGTAGVHSQVQLQQSGPEVVKPGASVKMSCKASGYTFTDHVISWVKQRTGQGLEWIGQIYPGSDNSYYSEKLKDKATLTADKSSNTAYMQLVSLTSEDSAVYFCAREGYGYGKNGVGYAMDYWGQGTSVTVSS

SEQ ID NO: 16 - protein, 127 aa, 2 Ambystoma laterale x Ambystoma jeffersonianum
MKSQTQVFVFLLLCVSGAHGSIVMTQTPKFLLVSAGDRVTITCKASQSVSNDVVWYQQKPGQSPKLLIYYASNRYTGVPDRFTGSGYGTDFTFTISTAQAEDLAVYFCQQDYSSPWTFGGGTKLEIK

SEQ ID NO: 17 - protein, 137 aa, 2 Ambystoma laterale x Ambystoma jeffersonianum
MGWSWVFLFLLSVTAGVHSQVQLVQSGAEVKKPGASVKLSCKASGYTFTSFDINWVRQAPEQRLEWMGWIFPGDGNTKYSQKFQGRATITRDTSASTAYMELSSLRSEDTAVYYCVRGEALYYFDYWGQGTLVTVSS

SEQ ID NO: 18 - protein, 126 aa, 2 Ambystoma laterale x Ambystoma jeffersonianum
MRPSIQFLGLLLFWLHGAQCDIQMTQSPSSLSASVGDRVTITCRASQDINKYLAWYQQKPGKVPKLLIYSTSTLQSGVPSRFSGSGSGTDFTLTISSLQPEDVATYYCLQYDDLFTFGQGTKLEIK

SEQ ID NO: 19 - protein, 143 aa, 2 Ambystoma laterale x Ambystoma jeffersonianum
MEWRIFLFILSGTAGVHSQVQLVQSGAEVKKPGASVKVSCKASGYTFTDHVISWVRQATGQGLEWMGQIYPGSDNSYYAQKFQGRVTLTADKSINTAYMELSSLRSEDTAVYYCAREGYGYGKNGVGYAMDYWGQGTLVTVSS

SEQ ID NO: 20 - protein, 127 aa, 2 Ambystoma laterale x Ambystoma jeffersonianum
MKSQTQVFVFLLLCVSGAHGDIVMTQSPDSLAVSLGERATINCKASQSVSNDVVWYQQKPGQPPKLLIYYASNRYTGVPDRFSGSGYGTDFTLTISSLQAEDVAVYYCQQDYSSPWTFGGGTKVEIK

SEQ ID NO: 21 - DNA, 24 bp, 2 Ambystoma laterale x Ambystoma jeffersonianum
ggctacaccttcacaagctttgat

SEQ ID NO: 22 - DNA, 21 bp, 2 Ambystoma laterale x Ambystoma jeffersonianum
atttttcctggagatggtaat

SEQ ID NO: 23 - DNA, 33 bp, 2 Ambystoma laterale x Ambystoma jeffersonianum
gtaagaggggaggccctgtattactttgactac

SEQ ID NO: 24 - DNA, 24 bp, 2 Ambystoma laterale x Ambystoma jeffersonianum
ggatacacattcactgaccatgtc

SEQ ID NO: 25 - DNA, 24 bp, 2 Ambystoma laterale x Ambystoma jeffersonianum
atttatcctggaagtgataatagt

SEQ ID NO: 26 - DNA, 54 bp, 2 Ambystoma laterale x Ambystoma jeffersonianum
gcaagagagggctatggttatggaaaaaacggagttggctatgctatggactac

SEQ ID NO: 27 - DNA, 18 bp, 2 Ambystoma laterale x Ambystoma jeffersonianum
caagacattaataagtat

SEQ ID NO: 28 - DNA, 9 bp, 2 Ambystoma laterale x Ambystoma jeffersonianum
tccacatct

SEQ ID NO: 29 - DNA, 24 bp, 2 Ambystoma laterale x Ambystoma jeffersonianum
ctgcagtatgatgatctattcacg

SEQ ID NO: 30 - DNA, 18 bp, 2 Ambystoma laterale x Ambystoma jeffersonianum
cagagtgtgagtaatgat

SEQ ID NO: 31 - DNA, 9 bp, 2 Ambystoma laterale x Ambystoma jeffersonianum
tatgcatcc

SEQ ID NO: 32 - DNA, 27 bp, 2 Ambystoma laterale x Ambystoma jeffersonianum
cagcaggattattcctctccgtggacg

SEQ ID NO: 33 - DNA, 411 bp, 2 Ambystoma laterale x Ambystoma jeffersonianum
atgggatggagctgggtctttctcttcctcctgtcagtaactgcaggtgtccactcccaggttcagctgcagcagtctggagctgaactggtaaagcctggggcttcagtgaagttgtcctgcaaggcttctggctacaccttcacaagctttgatataaactgggtgaggcagaggcctgaacagggacttgagtggattggatggatttttcctggagatggtaatactaagtccaatgagaaatttaagggcaaggccacactgactacagacaaatcctccagcacagcctacatgcagctcagcaggctgacatctgaggactctgctgtctatttctgtgtaagaggggaggccctgtattactttgactactggggcccaggcaccactctcacagtctcctca

SEQ ID NO: 34 - DNA, 379 bp, 2 Ambystoma laterale x Ambystoma jeffersonianum
atgagaccgtctattcagttcctggggctcttgttgttctggcttcatggtgctcagtgtgacatccagatgacacagtctccatcctcactgtctgcatctctgggaggcaaagtcaccatcacttgcaagccaagccaagacattaataagtatatagcttggtaccaacacaagcctggaaaaggtcctaggctgctcatacattccacatctacattacagccaggcatcccatcaaggttcagtggaagtgggtctgggagagattattccttcaccatcagcaacctggaacctgaagatattgcaacttattattgtctgcagtatgatgatctattcacgttcggctcggggacaaagttggaaataaaac

SEQ ID NO: 35 - DNA, 429 bp, 2 Ambystoma laterale x Ambystoma jeffersonianum
atggaatggaggatctttctcttcatcctgtcaggaactgcaggtgtccactcccaggttcagctgcagcagtctggacctgaggtggtgaagcctggggcttcagtgaagatgtcctgcaaggcttctggatacacattcactgaccatgtcataagctgggtgaagcagagaactggacagggccttgagtggattggacagatttatcctggaagtgataatagttactacagtgagaagttgaaggacaaggccacactgactgcagacaaatcctccaacacagcctacatgcagctcgtcagcctgacatctgaggactctgcggtctatttctgtgcaagagagggctatggttatggaaaaaacggagttggctatgctatggactactggggtcaaggaacctcagtcaccgtctcctca

SEQ ID NO: 36 - DNA, 382 bp, 2 Ambystoma laterale x Ambystoma jeffersonianum
atgaagtcacagacccaggtcttcgtatttctactgctctgtgtgtctggtgctcatgggagtattgtgatgacccagactcccaaattcctgcttgtatcagcaggagacagggttaccataacctgcaaggccagtcagagtgtgagtaatgatgtagtttggtaccaacagaagccagggcagtctcctaaactgctgatatactatgcatccaatcgctacactggagtccctgatcgcttcaccggcagtggatatgggacggatttcactttcaccatcagcactgcgcaggctgaagacctggcagtttatttctgtcagcaggattattcctctccgtggacgttcggtgggggcaccaagctggaaatcaaac

SEQ ID NO: 37 - DNA, 412 bp, 2 Ambystoma laterale x Ambystoma jeffersonianum
atgggctggtcctgggtgttcctgttcctgctgagcgtgaccgccggcgtgcactcccaggtgcagctggtgcagtccggcgccgaggtgaagaagcccggcgcctccgtgaagctgagctgtaaggcctccggctacaccttcacctccttcgacattaactgggtgcggcaggcccccgagcagcgcctggagtggatgggctggatcttccccggcgacggcaacaccaagtactcccagaagttccagggaagagctaccatcaccagagatacatccgcttctacagcttacatggagctgtctagcctgagatctgaggatacagctgtgtattactgtgtgagaggagaggctctgtactattttgattattggggccagggcaccctggtgacagtgtcttctg

SEQ ID NO: 38 - DNA, 379 bp, 2 Ambystoma laterale x Ambystoma jeffersonianum
atgagaccttctatccagtttctgggcctgctgctgttttggctgcatggcgcccagtgcgatatccagatgacccagtctccatctagcctgtccgcttctgtgggcgatagagtgaccatcacatgcagagcttctcaggatatcaataagtatctggcttggtatcagcagaagcctggaaaggtgcctaagctgctgatctactctacatctaccctgcagtctggagtgccttctagattttctggatctggctctggcaccgattttacactgacaatctcttctctgcagcctgaggatgtggctacatattattgtctgcagtatgatgatctgttcacctttggccagggcaccaagctggagatcaagc

SEQ ID NO: 39 - DNA, 430 bp, 2 Ambystoma laterale x Ambystoma jeffersonianum
atggagtggagaatctttctgtttatcctgtctggcacagctggagtgcattctcaggtgcagctggtgcagtctggggccgaggtgaaaaagccaggcgcttctgtgaaggtgtcttgcaaggcctccggctacaccttcaccgaccacgtgatctcctgggtgcgccaggccaccggccagggcctggagtggatgggccagatctaccccggctccgacaactcctactacgcccagaagttccagggcagggtgactctgaccgccgacaagtccatcaacaccgcctacatggagctgtcctccctgaggtccgaggacaccgccgtgtactactgcgccagggagggctacggctacggcaagaacggcgtgggctacgccatggattattggggccagggcaccctggtgacagtgtcttctg

SEQ ID NO: 40 - DNA, 382 bp, 2 Ambystoma laterale x Ambystoma jeffersonianum
atgaagtctcagacccaggtgtttgtgtttctgctgctgtgtgtgtctggcgctcatggcgatatcgtgatgacacagtctcctgattctctggccgtgtctctgggcgaaagagctacaatcaactgtaaggcttctcagtctgtgtctaatgatgtggtgtggtaccagcagaagcctgggcagccccccaagctgctgatctactacgcctccaacaggtacaccggcgtgcccgacaggttctccggctccggctacggcaccgacttcaccctgaccatctcctccctgcaggccgaggacgtggccgtgtactactgccagcaggactactcctccccctggaccttcggcggcggcaccaaggtggagatcaagc